European Patent Application EP 4 317 415 A1, published February 7, 2024. Title: BACILLUS NATTO FOR PRODUCING MENAQUINONE-7 AND USE THEREOF. Applicant: Hubei Magic Health Technology Co.,Ltd. The sequence listing filed with the application follows.

SEQUENCE LISTING (1 sequence)

SEQ ID NO: 1 - DNA, 1398 bp, Bacillus natto
  source 1..1398: mol_type = other DNA
tgcaagtcgagcggacagatgggagcttgctccctgatgttagcggcggacgggtgagtaacacgtgggtaacctgcctgtaagactgggataactccgggaaaccggggctaataccggatggttgtttgaaccgcatggttcaaacataaaaggtggcttcggctaccacttacagatggacccgcggcgcattagctagttggtgaggtaacggctcaccaaggcaacgatgcgtagccgacctgagagggtgatcggccacactgggactgagacacggcccagactcctacgggaggcagcagtagggaatcttccgcaatggacgaaagtctgacggagcaacgccgcgtgagtgatgaaggttttcggatcgtaaagctctgttgttagggaagaacaagtaccgttcgaatagggcggtaccttgacggtacctaaccagaaagccacggctaactacgtgccagcagccgcggtaatacgtaggtggcaagcgttgtccggaattattgggcgtaaagggctcgcaggcggtttcttaagtctgatgtgaaagcccccggctcaaccggggagggtcattggaaactggggaacttgagtgcagaagaggagagtggaattccacgtgtagcggtgaaatgcgtagagatgtggaggaacaccagtggcgaaggcgactctctggtctgtaactgacgctgaggagcgaaagcgtggggagcgaacaggattagataccctggtagtccacgccgtaaacgatgagtgctaagtgttagggggtttccgcccctttagtgctgcagctaacgcattaagcactccgcctggggagtacggtcgcaagactgaaactcaaaggaattgacgggggcccgcacaagcggtggagcatgtggtttaattcgaagcaacgcgaagaaccttaccaggtcttgacatcctctgacaatcctagagataggacgtccccttcgggggcagagtgacaggtggtgcatggttgtcgtcagctcgtgtcgtgagatgttgggttaagtcccgcaacgagcgcaacccttgatcttagttgccagcattcagttgggcactctaaggtgactgccggtgacaaaccggaggaaggtggggatgacgtcaaatcatcatgccccttatgacctgggctacacacgtgctacaatggacagaacaaagggcagcgaaaccgcgaggttaagccaatcccacaaatctgttctcagttcggatcgcagtctgcaactcgactgcgtgaagctggaatcgctagtaatcgcggatcagcatgccgcggtgaatacgttcccgggccttgtacacaccgcccgtcacaccacgagagtttgtaacacccgaagtcggtgaggt